European Patent Specification EP 3 620 533 B1, published January 18, 2023. Title: CLOSED NUCLEIC ACID STRUCTURES. Applicant: Nelson, Norman C. Chelliserry, Jijumon Brentano, Steven T. Lyakhov, Dmitry Friedenberg, Matthew C. Shapiro, Anne-Laure. The sequence listing filed with the application follows.

SEQUENCE LISTING (14 sequences)

SEQ ID NO: 1 - DNA, 6 bp, Artificial Sequence
  Synthesized
gcgccg

SEQ ID NO: 2 - DNA, 6 bp, Artificial Sequence
  Synthesized
cggcgc

SEQ ID NO: 3 - DNA, 24 bp, Artificial Sequence
  Synthesized
gggccgtttcccggtcttaaaaaa

SEQ ID NO: 4 - DNA, 24 bp, Artificial Sequence
  Synthesized
tggttgtgtccgcatctgaaaaaa

SEQ ID NO: 5 - DNA, 63 bp, Artificial Sequence
  Synthesized
aagaccgggaaacggcccatctctctcttttcctcctcctccgttgttgttgttgagagagat

SEQ ID NO: 6 - DNA, 63 bp, Artificial Sequence
  Synthesized
cagatgcggacacaaccaatctctctcttttcctcctcctccgttgttgttgttgagagagat

SEQ ID NO: 7 - DNA, 17 bp, Artificial Sequence
  Synthesized
gtaaaacgacggccagt

SEQ ID NO: 8 - DNA, 19 bp, Artificial Sequence
  Synthesized
ggaaacagctatgaccatg

SEQ ID NO: 9 - DNA, 24 bp, Artificial Sequence
  Synthesized
  misc_feature 24: C = reverse polarity nucleotide
taatccgtaaaacgacggccagtc

SEQ ID NO: 10 - DNA, 26 bp, Artificial Sequence
  Synthesized
  misc_feature 26: C = reverse polarity nucleotide
taatccggaaacagctatgaccatgc

SEQ ID NO: 11 - DNA, 49 bp, Artificial Sequence
  Synthesized
tctctctcttttcctcctcctccgttgttgttgttgagagagataatcc

SEQ ID NO: 12 - DNA, 6 bp, Artificial Sequence
  Synthesized
taatcc

SEQ ID NO: 13 - DNA, 10 bp, Artificial Sequence
  Synthesized
ttcgcggcaa

SEQ ID NO: 14 - DNA, 10 bp, Artificial Sequence
  Synthesized
ttgccgcgaa